European Patent Application EP 4 574 846 A1, published June 25, 2025. Title: ANTI-VEGFA FUSION PROTEIN, AND PREPARATION METHOD THEREOF AND USE THEREOF. Applicant: Quaerite Biopharm Research (Beijing) Co., Ltd. The sequence listing filed with the application follows.

SEQUENCE LISTING (159 sequences)

SEQ ID NO: 1 - protein, 5 aa, synthetic construct
SYTMG

SEQ ID NO: 2 - protein, 16 aa, synthetic construct
  SITE 10..11: note = XX can be DS, DA, NT, DT, NA or NS
AISKGGYKYXXVSLEA

SEQ ID NO: 3 - protein, 17 aa, synthetic construct
  SITE 10: note = R or K
  SITE 13: note = D, N, E or K
TRAYGSSRLXLAXTYEY

SEQ ID NO: 4 - protein, 16 aa, synthetic construct
AISKGGYKYDSVSLEA

SEQ ID NO: 5 - protein, 16 aa, synthetic construct
AISKGGYKYDAVSLEA

SEQ ID NO: 6 - protein, 16 aa, synthetic construct
AISKGGYKYNTVSLEA

SEQ ID NO: 7 - protein, 16 aa, synthetic construct
AISKGGYKYDTVSLEA

SEQ ID NO: 8 - protein, 16 aa, synthetic construct
AISKGGYKYNAVSLEA

SEQ ID NO: 9 - protein, 17 aa, synthetic construct
TRAYGSSRLRLADTYEY

SEQ ID NO: 10 - protein, 17 aa, synthetic construct
TRAYGSSRLRLANTYEY

SEQ ID NO: 11 - protein, 17 aa, synthetic construct
TRAYGSSRLRLAETYEY

SEQ ID NO: 12 - protein, 17 aa, synthetic construct
TRAYGSSRLRLAKTYEY

SEQ ID NO: 13 - protein, 125 aa, synthetic construct
QLQLVESGGGSVQPGGSLRLSCEVSGRTFSSYTMGWFRQAPGKEREFVVAISKGGYKYDSVSLEARFTISKDNTKNTVYLQMNSLKPEDTAVYYCAATRAYGSSRLRLADTYEYWGQGTQVTVSS

SEQ ID NO: 14 - protein, 125 aa, synthetic construct
QLQLVESGGGSVQPGGSLRLSCEVSGRTFSSYTMGWFRQAPGKEREFVVAISKGGYKYDTVSLEARFTISKDNTKNTVYLQMNSLKPEDTAVYYCAGTRAYGSSRLKLADTYEYWGQGTQVTVSS

SEQ ID NO: 15 - protein, 125 aa, synthetic construct
QLQLVESGGGSVQPGGSLRLSCEVSGRTFSSYTMGWFRQAPGKEREFVVAISKGGYKYNTVSLEARFTISKDNTKNTVYLQMNSLKPEDTAVYYCAGTRAYGSSRLKLAETYEYWGQGTQVTVSS

SEQ ID NO: 16 - protein, 125 aa, synthetic construct
QLQLVESGGGSVQPGGSLRLSCEVSGRTFTSYTMGWFRQAPGKEREFVVAISKGGYKYDAVSLEARFTISKDNTKNTVYLQMNSLKPEDTAVYYCAGTRAYGSSRLRLADTYEYWGQGTQVTVSS

SEQ ID NO: 17 - protein, 125 aa, synthetic construct
QLQLVESGGGSVQPGGSLRLSCEVSGRTFTSYTMGWFRQAPGKEREFVVAISKGGYKYNTVSLEARFTISKDNTKNTVYLQMNSLKPEDTAVYYCAGTRAYGSSRLRLANTYEYWGQGTQVTVSS

SEQ ID NO: 18 - protein, 125 aa, synthetic construct
QLQLVESGGGSVQPGGSLRLSCEVSGRTFASYTMGWFRQAPGKEREFVVAISKGGYKYDSVSLEARFTISKDNTKNTVYLQMNSLKPEDTAVYYCAGTRAYGSSRLRLAETYEYWGQGTQVTVSS

SEQ ID NO: 19 - protein, 125 aa, synthetic construct
QLQLVESGGGSVQPGGSLRLSCEVSGRTFSSYTMGWFRQAPGKEREFVVAISKGGYKYDTVSLEARFTISKDNTKNTVYLQMNSLKPEDTAVYYCAATRAYGSSRLRLAKTYEYWGQGTQVTVSS

SEQ ID NO: 20 - protein, 125 aa, synthetic construct
QLQLVESGGGSVQPGGSLRLSCEVSGRTFSSYTMGWFRQAPGKEREFVVAISKGGYKYNSVSLEARFTISKDNTKNTVYLQMNSLKPEDTAVYYCAGTRAYGSSRLRLADTYEYWGQGTQVTVSS

SEQ ID NO: 21 - protein, 125 aa, synthetic construct
QLQLVESGGGSVQPGGSLRLSCEVSGRTFSSYTMGWFRQAPGKEREFVVAISKGGYKYNSVSLEARFTISKDNTKNTVYLQMNSLKPEDTAVYYCAATRAYGSSRLKLANTYEYWGQGTQVTVSS

SEQ ID NO: 22 - protein, 125 aa, synthetic construct
QLQLVESGGGSVQPGGSLRLSCEVSGRTFTSYTMGWFRQAPGKEREFVVAISKGGYKYNTVSLEARFTISKDNTKNTVYLQMNSLKPEDTAVYYCAGTRAYGSSRLRLAETYEYWGQGTQVTVSS

SEQ ID NO: 23 - protein, 125 aa, synthetic construct
QLQLVESGGGSVQPGGSLRLSCEVSGRTFSSYTMGWFRQAPGKEREFVVAISKGGYKYDSVSLEARFTISKDNTKNTVYLQMNSLKPEDTAVYYCAATRAYGSSRLKLADTYEYWGQGTQVTVSS

SEQ ID NO: 24 - protein, 125 aa, synthetic construct
QLQLVESGGGSVQPGGSLRLSCEVSGRTFTSYTMGWFRRAPGKEREFVVAISKGGYKYDSVSLEARFTISKDNTKNTVYLQMNSLKPEDTAVYYCAGTRAYGSSRLKLAKTYEYWGQGTQVTVSS

SEQ ID NO: 25 - protein, 125 aa, synthetic construct
QLQLVESGGGSVQPGGSLRLSCEVSGRTFSSYTMGWFRQAPGKEREFVVAISKGGYKYDSVSLEARFTISKDNTKNTVYLQMNSLKPEDTAVYYCAGTRAYGSSRLRLANTYEYWGQGTQVTVSS

SEQ ID NO: 26 - protein, 125 aa, synthetic construct
QLQLVESGGGSVQPGGSLRLSCEVSGRTFSSYTMGWFRQAPGKGREFVVAISKGGYKYDAVSLEARFTISKDNTKNTVYLQMNSLKPEDTAVYYCAATRAYGSSRLRLAKTYEYWGQGTQVTVSS

SEQ ID NO: 27 - protein, 125 aa, synthetic construct
QLQLVESGGGSVQPGGSLRLSCEVSGRTFASYTMGWFRQAPGKEREFVVAISKGGYKYDAVSLEARFTISKDNTKNTVYLQMNSLKPEDTAVYYCAGTRAYGSSRLRLAKTYEYWGQGTQVTVSS

SEQ ID NO: 28 - protein, 125 aa, synthetic construct
QLQLVESGGGSVQPGGSLRLSCEVSGRTFSSYTMGWFRQAPGKEREFVVAISKGGYKYDSVSLEARFTISKDNTKNTVYLQMNSLKPEDTAVYYCAATRAYGSSRLRLAKTYEYWGQGTQVTVSS

SEQ ID NO: 29 - protein, 125 aa, synthetic construct
QLQLVESGGGSVQPGGSLRLSCEVSGRTFASYTMGWFRQAPGKEREFVVAISKGGYKYDSVSLEARFTISKDNTKNTVYLQMNSLKPEDTAVYYCAGTRAYGSSRLRLADTYEYWGQGTQVTVSS

SEQ ID NO: 30 - protein, 125 aa, synthetic construct
QLQLVESGGGSVQPGGSLRLSCEVSGRTFTSYTMGWFRQAPGKEREFVVAISKGGYKYNAVSLEARFTISKDNTKNTVYLQMNSLKPEDTAVYYCAGTRAYGSSRLRLAKTYEYWGQGTQVTVSS

SEQ ID NO: 31 - protein, 125 aa, synthetic construct
QLQLVESGGGSVQPGGSLRLSCEVSGRTFSSYTMGWFRQAPGKEREFVVAISKGGYKYDSVSLEARFTISKDNTKNTVYLQMNSLKPEDTAVYYCAGTRAYGSSRLRLAKTYEYWGQGTQVTVSS

SEQ ID NO: 32 - protein, 125 aa, synthetic construct
QLQLVESGGGSVQPGGSLRLSCEVSGRTFTSYTMGWFRQAPGKEREFVVAISKGGYKYDSVSLEARFTISKDNTKNTVYLQMNSLKPEDTAVYYCAGTRAYGSSRLRLANTYEYWGQGTQVTVSS

SEQ ID NO: 33 - protein, 16 aa, synthetic construct
AISKGGYKYNSVSLEA

SEQ ID NO: 34 - protein, 17 aa, synthetic construct
TRAYGSSRLKLANTYEY

SEQ ID NO: 35 - protein, 125 aa, synthetic construct
EVQLVESGGGLVQPGGSLRLSCAASGRTFSSYTMGWFRQAPGKEREFVVAISKGGYKYDSVSLEARFTISRDNSKNTVYLQMNSLRAEDTAVYYCAATRAYGSSRLRLADTYEYWGQGTLVTVSS

SEQ ID NO: 36 - protein, 125 aa, synthetic construct
EVQLVESGGGLVQPGGSLRLSCAASGRTFSSYTMGWFRQAPGKEREFVVAISKGGYKYDSVSLEARFTISRDNSKNTLYLQMNSLRPEDTAVYYCAATRAYGSSRLRLADTYEYWGQGTLVTVSS

SEQ ID NO: 37 - protein, 125 aa, synthetic construct
EVQLVESGGGLVQPGGSLRLSCAASGRTFSSYTMGWFRQAPGKEREFVVAISKGGYKYDSVSLEARFTISRDNSKNTVYLQMNSLRPEDTAVYYCAATRAYGSSRLRLADTYEYWGQGTLVTVSS

SEQ ID NO: 38 - protein, 125 aa, synthetic construct
EVQLVESGGGLVQPGGSLRLSCAASGRTFSSYTMGWFRQAPGKEREFVVAISKGGYKYDSVSLEARFTISRDNAKNTVYLQMNSLRPEDTAVYYCAATRAYGSSRLRLADTYEYWGQGTLVTVSS

SEQ ID NO: 39 - protein, 125 aa, synthetic construct
EVQLVESGGGLVQPGGSLRLSCAASGRTFSSYTMGWFRQAPGKEREFVVAISKGGYKYDSVSLEARFTISRDNAKNTVYLQMNSLRAEDTAVYYCASTRAYGSSRLRLADTYEYWGQGTLVTVSS

SEQ ID NO: 40 - protein, 125 aa, synthetic construct
EVQLVESGGGLVQPGGSLRLSCAASGRTFSSYTMGWFRQAPGKEREFVVAISKGGYKYDSVSLEARFTISRDNAKNTVYLQMNSLRPEDTAVYYCASTRAYGSSRLRLADTYEYWGQGTLVTVSS

SEQ ID NO: 41 - protein, 125 aa, synthetic construct
EVQLVESGGGLVQPGGSLRLSCAVSGRTFSSYTMGWFRQAPGKEREFVVAISKGGYKYDSVSLEARFTISRDNAKNTVYLQMNSLRPEDTAVYYCAATRAYGSSRLRLADTYEYWGQGTLVTVSS

SEQ ID NO: 42 - protein, 125 aa, synthetic construct
EVQLVESGGGLVQPGGSLRLSCAASGRTFSSYTMGWFRQAPGKEREFVVAISKGGYKYDSVSLEARFTISRDNAKNTVYLQMNSLRAEDTAVYYCAATRAYGSSRLRLADTYEYWGQGTLVTVSS

SEQ ID NO: 43 - protein, 125 aa, synthetic construct
EVQLVESGGGLVQPGGSLRLSCAVSGRTFSSYTMGWFRQAPGKEREFVVAISKGGYKYDSVSLEARFTISRDNSKNTVYLQMNSLRPEDTAVYYCAATRAYGSSRLRLADTYEYWGQGTLVTVSS

SEQ ID NO: 44 - protein, 125 aa, synthetic construct
EVQLVESGGGLVQPGGSLRLSCAASGRTFTSYTMGWFRQAPGKEREFVVAISKGGYKYDAVSLEARFTISRDNSKNTVYLQMNSLRPEDTAVYYCAGTRAYGSSRLRLADTYEYWGQGTLVTVSS

SEQ ID NO: 45 - protein, 125 aa, synthetic construct
EVQLVESGGGLVQPGGSLRLSCAASGRTFTSYTMGWFRQAPGKEREFVVAISKGGYKYDAVSLEARFTISRDNAKNTVYLQMNSLRPEDTAVYYCAGTRAYGSSRLRLADTYEYWGQGTLVTVSS

SEQ ID NO: 46 - protein, 125 aa, synthetic construct
EVQLVESGGGLVQPGGSLRLSCAASGRTFASYTMGWFRQAPGKEREFVVAISKGGYKYDSVSLEARFTISRDNSKNTVYLQMNSLRPEDTAVYYCAGTRAYGSSRLRLAETYEYWGQGTLVTVSS

SEQ ID NO: 47 - protein, 125 aa, synthetic construct
EVQLVESGGGLVQPGGSLRLSCAASGRTFASYTMGWFRQAPGKEREFVVAISKGGYKYDSVSLEARFTISRDNAKNTVYLQMNSLRPEDTAVYYCAGTRAYGSSRLRLAETYEYWGQGTLVTVSS

SEQ ID NO: 48 - protein, 125 aa, synthetic construct
EVQLVESGGGLVQPGGSLRLSCAASGRTFSSYTMGWFRQAPGKEREFVVAISKGGYKYDAVSLEARFTISRDNSKNTVYLQMNSLRAEDTAVYYCAATRAYGSSRLRLAKTYEYWGQGTLVTVSS

SEQ ID NO: 49 - protein, 125 aa, synthetic construct
EVQLVESGGGLVQPGGSLRLSCAASGRTFSSYTMGWFRQAPGKEREFVVAISKGGYKYDAVSLEARFTISRDNSKNTLYLQMNSLRPEDTAVYYCAATRAYGSSRLRLAKTYEYWGQGTLVTVSS

SEQ ID NO: 50 - protein, 125 aa, synthetic construct
EVQLVESGGGLVQPGGSLRLSCAASGRTFSSYTMGWFRQAPGKEREFVVAISKGGYKYDAVSLEARFTISRDNSKNTVYLQMNSLRPEDTAVYYCAATRAYGSSRLRLAKTYEYWGQGTLVTVSS

SEQ ID NO: 51 - protein, 125 aa, synthetic construct
EVQLVESGGGLVQPGGSLRLSCAASGRTFSSYTMGWFRQAPGKGREFVVAISKGGYKYDAVSLEARFTISRDNSKNTVYLQMNSLRPEDTAVYYCAATRAYGSSRLRLAKTYEYWGQGTLVTVSS

SEQ ID NO: 52 - protein, 125 aa, synthetic construct
EVQLVESGGGLVQPGGSLRLSCAASGRTFSSYTMGWFRQAPGKEREFVVAISKGGYKYNAVSLEARFTISRDNSKNTVYLQMNSLRPEDTAVYYCAATRAYGSSRLRLAKTYEYWGQGTLVTVSS

SEQ ID NO: 53 - protein, 125 aa, synthetic construct
EVQLVESGGGLVQPGGSLRLSCAASGRTFSSYTMGWFRQAPGKEREFVVAISKGGYKYNAVSLEARFTISRDNAKNTVYLQMNSLRPEDTAVYYCASTRAYGSSRLRLAKTYEYWGQGTLVTVSS

SEQ ID NO: 54 - protein, 125 aa, synthetic construct
EVQLVESGGGLVQPGGSLRLSCAASGRTFTSYTMGWFRQAPGKEREFVVAISKGGYKYNAVSLEARFTISRDNSKNTVYLQMNSLRPEDTAVYYCAATRAYGSSRLRLAKTYEYWGQGTLVTVSS

SEQ ID NO: 55 - protein, 125 aa, synthetic construct
EVQLVESGGGLVQPGGSLRLSCAASGRTFTSYTMGWFRQAPGKEREFVVAISKGGYKYNAVSLEARFTISRDNAKNTVYLQMNSLRPEDTAVYYCASTRAYGSSRLRLAKTYEYWGQGTLVTVSS

SEQ ID NO: 56 - protein, 125 aa, synthetic construct
EVQLVESGGGLVQPGGSLRLSCAASGRTFSSYTMGWFRQAPGKEREFVVAISKGGYKYDSVSLEARFTISRDNSKNTVYLQMNSLRAEDTAVYYCAATRAYGSSRLRLANTYEYWGQGTLVTVSS

SEQ ID NO: 57 - protein, 125 aa, synthetic construct
EVQLVESGGGLVQPGGSLRLSCAASGRTFSSYTMGWFRQAPGKEREFVVAISKGGYKYDSVSLEARFTISRDNSKNTLYLQMNSLRPEDTAVYYCAATRAYGSSRLRLANTYEYWGQGTLVTVSS

SEQ ID NO: 58 - protein, 125 aa, synthetic construct
EVQLVESGGGLVQPGGSLRLSCAASGRTFSSYTMGWFRQAPGKEREFVVAISKGGYKYDSVSLEARFTISRDNSKNTVYLQMNSLRPEDTAVYYCAATRAYGSSRLRLANTYEYWGQGTLVTVSS

SEQ ID NO: 59 - protein, 125 aa, synthetic construct
EVQLVESGGGLVQPGGSLRLSCAASGRTFTSYTMGWFRQAPGKEREFVVAISKGGYKYDSVSLEARFTISRDNSKNTVYLQMNSLRAEDTAVYYCAGTRAYGSSRLRLANTYEYWGQGTLVTVSS

SEQ ID NO: 60 - protein, 125 aa, synthetic construct
EVQLVESGGGLVQPGGSLRLSCAASGRTFTSYTMGWFRQAPGKEREFVVAISKGGYKYDSVSLEARFTISRDNSKNTLYLQMNSLRPEDTAVYYCAGTRAYGSSRLRLANTYEYWGQGTLVTVSS

SEQ ID NO: 61 - protein, 125 aa, synthetic construct
EVQLVESGGGLVQPGGSLRLSCAASGRTFTSYTMGWFRQAPGKEREFVVAISKGGYKYDSVSLEARFTISRDNAKNTVYLQMNSLRPEDTAVYYCAGTRAYGSSRLRLANTYEYWGQGTLVTVSS

SEQ ID NO: 62 - protein, 259 aa, synthetic construct
QLQLVESGGGSVQPGGSLRLSCEVSGRTFSSYTMGWFRQAPGKEREFVVAISKGGYKYDSVSLEARFTISKDNTKNTVYLQMNSLKPEDTAVYYCAATRAYGSSRLRLADTYEYWGQGTQVTVSSGGGGSGGGSQLQLVESGGGSVQPGGSLRLSCEVSGRTFSSYTMGWFRQAPGKEREFVVAISKGGYKYDSVSLEARFTISKDNTKNTVYLQMNSLKPEDTAVYYCAATRAYGSSRLRLADTYEYWGQGTQVTVSS

SEQ ID NO: 63 - protein, 259 aa, synthetic construct
QLQLVESGGGSVQPGGSLRLSCEVSGRTFASYTMGWFRQAPGKEREFVVAISKGGYKYDSVSLEARFTISKDNTKNTVYLQMNSLKPEDTAVYYCAGTRAYGSSRLRLAETYEYWGQGTQVTVSSGGGGSGGGSQLQLVESGGGSVQPGGSLRLSCEVSGRTFASYTMGWFRQAPGKEREFVVAISKGGYKYDSVSLEARFTISKDNTKNTVYLQMNSLKPEDTAVYYCAGTRAYGSSRLRLAETYEYWGQGTQVTVSS

SEQ ID NO: 64 - protein, 259 aa, synthetic construct
QLQLVESGGGSVQPGGSLRLSCEVSGRTFSSYTMGWFRQAPGKEREFVVAISKGGYKYDSVSLEARFTISKDNTKNTVYLQMNSLKPEDTAVYYCAGTRAYGSSRLRLANTYEYWGQGTQVTVSSGGGGSGGGSQLQLVESGGGSVQPGGSLRLSCEVSGRTFSSYTMGWFRQAPGKEREFVVAISKGGYKYDSVSLEARFTISKDNTKNTVYLQMNSLKPEDTAVYYCAGTRAYGSSRLRLANTYEYWGQGTQVTVSS

SEQ ID NO: 65 - protein, 259 aa, synthetic construct
QLQLVESGGGSVQPGGSLRLSCEVSGRTFSSYTMGWFRQAPGKGREFVVAISKGGYKYDAVSLEARFTISKDNTKNTVYLQMNSLKPEDTAVYYCAATRAYGSSRLRLAKTYEYWGQGTQVTVSSGGGGSGGGSQLQLVESGGGSVQPGGSLRLSCEVSGRTFSSYTMGWFRQAPGKGREFVVAISKGGYKYDAVSLEARFTISKDNTKNTVYLQMNSLKPEDTAVYYCAATRAYGSSRLRLAKTYEYWGQGTQVTVSS

SEQ ID NO: 66 - protein, 259 aa, synthetic construct
QLQLVESGGGSVQPGGSLRLSCEVSGRTFASYTMGWFRQAPGKEREFVVAISKGGYKYDAVSLEARFTISKDNTKNTVYLQMNSLKPEDTAVYYCAGTRAYGSSRLRLAKTYEYWGQGTQVTVSSGGGGSGGGSQLQLVESGGGSVQPGGSLRLSCEVSGRTFASYTMGWFRQAPGKEREFVVAISKGGYKYDAVSLEARFTISKDNTKNTVYLQMNSLKPEDTAVYYCAGTRAYGSSRLRLAKTYEYWGQGTQVTVSS

SEQ ID NO: 67 - protein, 259 aa, synthetic construct
QLQLVESGGGSVQPGGSLRLSCEVSGRTFSSYTMGWFRQAPGKEREFVVAISKGGYKYDSVSLEARFTISKDNTKNTVYLQMNSLKPEDTAVYYCAATRAYGSSRLRLAKTYEYWGQGTQVTVSSGGGGSGGGSQLQLVESGGGSVQPGGSLRLSCEVSGRTFSSYTMGWFRQAPGKEREFVVAISKGGYKYDSVSLEARFTISKDNTKNTVYLQMNSLKPEDTAVYYCAATRAYGSSRLRLAKTYEYWGQGTQVTVSS

SEQ ID NO: 68 - protein, 259 aa, synthetic construct
QLQLVESGGGSVQPGGSLRLSCEVSGRTFASYTMGWFRQAPGKEREFVVAISKGGYKYDSVSLEARFTISKDNTKNTVYLQMNSLKPEDTAVYYCAGTRAYGSSRLRLADTYEYWGQGTQVTVSSGGGGSGGGSQLQLVESGGGSVQPGGSLRLSCEVSGRTFASYTMGWFRQAPGKEREFVVAISKGGYKYDSVSLEARFTISKDNTKNTVYLQMNSLKPEDTAVYYCAGTRAYGSSRLRLADTYEYWGQGTQVTVSS

SEQ ID NO: 69 - protein, 259 aa, synthetic construct
QLQLVESGGGSVQPGGSLRLSCEVSGRTFSSYTMGWFRQAPGKEREFVVAISKGGYKYDSVSLEARFTISKDNTKNTVYLQMNSLKPEDTAVYYCAGTRAYGSSRLRLAKTYEYWGQGTQVTVSSGGGGSGGGSQLQLVESGGGSVQPGGSLRLSCEVSGRTFSSYTMGWFRQAPGKEREFVVAISKGGYKYDSVSLEARFTISKDNTKNTVYLQMNSLKPEDTAVYYCAGTRAYGSSRLRLAKTYEYWGQGTQVTVSS

SEQ ID NO: 70 - protein, 259 aa, synthetic construct
QLQLVESGGGSVQPGGSLRLSCEVSGRTFTSYTMGWFRQAPGKEREFVVAISKGGYKYDSVSLEARFTISKDNTKNTVYLQMNSLKPEDTAVYYCAGTRAYGSSRLRLANTYEYWGQGTQVTVSSGGGGSGGGSQLQLVESGGGSVQPGGSLRLSCEVSGRTFTSYTMGWFRQAPGKEREFVVAISKGGYKYDSVSLEARFTISKDNTKNTVYLQMNSLKPEDTAVYYCAGTRAYGSSRLRLANTYEYWGQGTQVTVSS

SEQ ID NO: 71 - protein, 259 aa, synthetic construct
QLQLVESGGGSVQPGGSLRLSCEVSGRTFSSYTMGWFRQAPGKEREFVVAISKGGYKYDSVSLEARFTISKDNTKNTVYLQMNSLKPEDTAVYYCAATRAYGSSRLRLADTYEYWGQGTQVTVSSGGGGSGGGSQLQLVESGGGSVQPGGSLRLSCEVSGRTFASYTMGWFRQAPGKEREFVVAISKGGYKYDSVSLEARFTISKDNTKNTVYLQMNSLKPEDTAVYYCAGTRAYGSSRLRLAETYEYWGQGTQVTVSS

SEQ ID NO: 72 - protein, 259 aa, synthetic construct
QLQLVESGGGSVQPGGSLRLSCEVSGRTFSSYTMGWFRQAPGKEREFVVAISKGGYKYDSVSLEARFTISKDNTKNTVYLQMNSLKPEDTAVYYCAATRAYGSSRLRLADTYEYWGQGTQVTVSSGGGGSGGGSQLQLVESGGGSVQPGGSLRLSCEVSGRTFSSYTMGWFRQAPGKGREFVVAISKGGYKYDAVSLEARFTISKDNTKNTVYLQMNSLKPEDTAVYYCAATRAYGSSRLRLAKTYEYWGQGTQVTVSS

SEQ ID NO: 73 - protein, 259 aa, synthetic construct
QLQLVESGGGSVQPGGSLRLSCEVSGRTFSSYTMGWFRQAPGKEREFVVAISKGGYKYDSVSLEARFTISKDNTKNTVYLQMNSLKPEDTAVYYCAATRAYGSSRLRLADTYEYWGQGTQVTVSSGGGGSGGGSQLQLVESGGGSVQPGGSLRLSCEVSGRTFTSYTMGWFRQAPGKEREFVVAISKGGYKYNAVSLEARFTISKDNTKNTVYLQMNSLKPEDTAVYYCAATRAYGSSRLRLAKTYEYWGQGTQVTVSS

SEQ ID NO: 74 - protein, 259 aa, synthetic construct
QLQLVESGGGSVQPGGSLRLSCEVSGRTFASYTMGWFRQAPGKEREFVVAISKGGYKYDSVSLEARFTISKDNTKNTVYLQMNSLKPEDTAVYYCAGTRAYGSSRLRLAETYEYWGQGTQVTVSSGGGGSGGGSQLQLVESGGGSVQPGGSLRLSCEVSGRTFSSYTMGWFRQAPGKGREFVVAISKGGYKYDAVSLEARFTISKDNTKNTVYLQMNSLKPEDTAVYYCAATRAYGSSRLRLAKTYEYWGQGTQVTVSS

SEQ ID NO: 75 - protein, 259 aa, synthetic construct
QLQLVESGGGSVQPGGSLRLSCEVSGRTFASYTMGWFRQAPGKEREFVVAISKGGYKYDSVSLEARFTISKDNTKNTVYLQMNSLKPEDTAVYYCAGTRAYGSSRLRLAETYEYWGQGTQVTVSSGGGGSGGGSQLQLVESGGGSVQPGGSLRLSCEVSGRTFTSYTMGWFRQAPGKEREFVVAISKGGYKYNAVSLEARFTISKDNTKNTVYLQMNSLKPEDTAVYYCAATRAYGSSRLRLAKTYEYWGQGTQVTVSS

SEQ ID NO: 76 - protein, 259 aa, synthetic construct
QLQLVESGGGSVQPGGSLRLSCEVSGRTFSSYTMGWFRQAPGKGREFVVAISKGGYKYDAVSLEARFTISKDNTKNTVYLQMNSLKPEDTAVYYCAATRAYGSSRLRLAKTYEYWGQGTQVTVSSGGGGSGGGSQLQLVESGGGSVQPGGSLRLSCEVSGRTFTSYTMGWFRQAPGKEREFVVAISKGGYKYNAVSLEARFTISKDNTKNTVYLQMNSLKPEDTAVYYCAATRAYGSSRLRLAKTYEYWGQGTQVTVSS

SEQ ID NO: 77 - skipped

SEQ ID NO: 78 - protein, 9 aa, synthetic construct
GGGGSGGGS

SEQ ID NO: 79 - protein, 9 aa, synthetic construct
SSSSSSSSS

SEQ ID NO: 80 - protein, 20 aa, synthetic construct
SSSSSSSSSSSSSSSSSSSS

SEQ ID NO: 81 - protein, 20 aa, synthetic construct
GGGGSGGGSGGGSGGGSGGS

SEQ ID NO: 82 - protein, 25 aa, synthetic construct
GGGGSGGGSGGGSGGGSGGGSGGGS

SEQ ID NO: 83 - protein, 30 aa, synthetic construct
GGGGSGGGSGGGGSGGGSGGGSGGGSGGGS

SEQ ID NO: 84 - protein, 39 aa, synthetic construct
GGGGSGGGSGGGGSGGGGSGGGGSGGGGSGGGGSGGGGS

SEQ ID NO: 85 - protein, 37 aa, synthetic construct
GSTSGSGKPGSGEGSTKGGSTSGSGKPGSGEGSTKGS

SEQ ID NO: 86 - protein, 17 aa, synthetic construct
PDSAPAPAPAPAPDGSS

SEQ ID NO: 87 - protein, 27 aa, synthetic construct
PDSAPAPAPAPAPAPAPAPAPAPDGSS

SEQ ID NO: 88 - protein, 30 aa, synthetic construct
LAEAAAKEAAAKEAAAKEAAAKEAAAKAAA

SEQ ID NO: 89 - protein, 33 aa, synthetic construct
PDSEAAAKEAAAKEAAAKEAAAKEAAAKPDGSS

SEQ ID NO: 90 - skipped

SEQ ID NO: 91 - protein, 6 aa, synthetic construct
AAAAAA

SEQ ID NO: 92 - protein, 250 aa, synthetic construct
QLQLVESGGGSVQPGGSLRLSCEVSGRTFSSYTMGWFRQAPGKEREFVVAISKGGYKYDSVSLEARFTISKDNTKNTVYLQMNSLKPEDTAVYYCAATRAYGSSRLRLADTYEYWGQGTQVTVSSQLQLVESGGGSVQPGGSLRLSCEVSGRTFSSYTMGWFRQAPGKEREFVVAISKGGYKYDSVSLEARFTISKDNTKNTVYLQMNSLKPEDTAVYYCAATRAYGSSRLRLADTYEYWGQGTQVTVSS

SEQ ID NO: 93 - protein, 253 aa, synthetic construct
QLQLVESGGGSVQPGGSLRLSCEVSGRTFSSYTMGWFRQAPGKEREFVVAISKGGYKYDSVSLEARFTISKDNTKNTVYLQMNSLKPEDTAVYYCAATRAYGSSRLRLADTYEYWGQGTQVTVSSAAAQLQLVESGGGSVQPGGSLRLSCEVSGRTFSSYTMGWFRQAPGKEREFVVAISKGGYKYDSVSLEARFTISKDNTKNTVYLQMNSLKPEDTAVYYCAATRAYGSSRLRLADTYEYWGQGTQVTVSS

SEQ ID NO: 94 - protein, 256 aa, synthetic construct
QLQLVESGGGSVQPGGSLRLSCEVSGRTFSSYTMGWFRQAPGKEREFVVAISKGGYKYDSVSLEARFTISKDNTKNTVYLQMNSLKPEDTAVYYCAATRAYGSSRLRLADTYEYWGQGTQVTVSSAAAAAAQLQLVESGGGSVQPGGSLRLSCEVSGRTFSSYTMGWFRQAPGKEREFVVAISKGGYKYDSVSLEARFTISKDNTKNTVYLQMNSLKPEDTAVYYCAATRAYGSSRLRLADTYEYWGQGTQVTVSS

SEQ ID NO: 95 - protein, 253 aa, synthetic construct
QLQLVESGGGSVQPGGSLRLSCEVSGRTFSSYTMGWFRQAPGKEREFVVAISKGGYKYDSVSLEARFTISKDNTKNTVYLQMNSLKPEDTAVYYCAATRAYGSSRLRLADTYEYWGQGTQVTVSSGGSQLQLVESGGGSVQPGGSLRLSCEVSGRTFSSYTMGWFRQAPGKEREFVVAISKGGYKYDSVSLEARFTISKDNTKNTVYLQMNSLKPEDTAVYYCAATRAYGSSRLRLADTYEYWGQGTQVTVSS

SEQ ID NO: 96 - protein, 280 aa, synthetic construct
QLQLVESGGGSVQPGGSLRLSCEVSGRTFSSYTMGWFRQAPGKEREFVVAISKGGYKYDSVSLEARFTISKDNTKNTVYLQMNSLKPEDTAVYYCAATRAYGSSRLRLADTYEYWGQGTQVTVSSGGGGSGGGSGGGGSGGGSGGGSGGGSGGGSQLQLVESGGGSVQPGGSLRLSCEVSGRTFSSYTMGWFRQAPGKEREFVVAISKGGYKYDSVSLEARFTISKDNTKNTVYLQMNSLKPEDTAVYYCAATRAYGSSRLRLADTYEYWGQGTQVTVSS

SEQ ID NO: 97 - protein, 289 aa, synthetic construct
QLQLVESGGGSVQPGGSLRLSCEVSGRTFSSYTMGWFRQAPGKEREFVVAISKGGYKYDSVSLEARFTISKDNTKNTVYLQMNSLKPEDTAVYYCAATRAYGSSRLRLADTYEYWGQGTQVTVSSGGGGSGGGSGGGGSGGGGSGGGGSGGGGSGGGGSGGGGSQLQLVESGGGSVQPGGSLRLSCEVSGRTFSSYTMGWFRQAPGKEREFVVAISKGGYKYDSVSLEARFTISKDNTKNTVYLQMNSLKPEDTAVYYCAATRAYGSSRLRLADTYEYWGQGTQVTVSS

SEQ ID NO: 98 - protein, 267 aa, synthetic construct
QLQLVESGGGSVQPGGSLRLSCEVSGRTFSSYTMGWFRQAPGKEREFVVAISKGGYKYDSVSLEARFTISKDNTKNTVYLQMNSLKPEDTAVYYCAATRAYGSSRLRLADTYEYWGQGTQVTVSSPDSAPAPAPAPAPDGSSQLQLVESGGGSVQPGGSLRLSCEVSGRTFSSYTMGWFRQAPGKEREFVVAISKGGYKYDSVSLEARFTISKDNTKNTVYLQMNSLKPEDTAVYYCAATRAYGSSRLRLADTYEYWGQGTQVTVSS

SEQ ID NO: 99 - protein, 277 aa, synthetic construct
QLQLVESGGGSVQPGGSLRLSCEVSGRTFSSYTMGWFRQAPGKEREFVVAISKGGYKYDSVSLEARFTISKDNTKNTVYLQMNSLKPEDTAVYYCAATRAYGSSRLRLADTYEYWGQGTQVTVSSPDSAPAPAPAPAPAPAPAPAPAPDGSSQLQLVESGGGSVQPGGSLRLSCEVSGRTFSSYTMGWFRQAPGKEREFVVAISKGGYKYDSVSLEARFTISKDNTKNTVYLQMNSLKPEDTAVYYCAATRAYGSSRLRLADTYEYWGQGTQVTVSS

SEQ ID NO: 100 - protein, 280 aa, synthetic construct
QLQLVESGGGSVQPGGSLRLSCEVSGRTFSSYTMGWFRQAPGKEREFVVAISKGGYKYDSVSLEARFTISKDNTKNTVYLQMNSLKPEDTAVYYCAATRAYGSSRLRLADTYEYWGQGTQVTVSSLAEAAAKEAAAKEAAAKEAAAKEAAAKAAAQLQLVESGGGSVQPGGSLRLSCEVSGRTFSSYTMGWFRQAPGKEREFVVAISKGGYKYDSVSLEARFTISKDNTKNTVYLQMNSLKPEDTAVYYCAATRAYGSSRLRLADTYEYWGQGTQVTVSS

SEQ ID NO: 101 - protein, 283 aa, synthetic construct
QLQLVESGGGSVQPGGSLRLSCEVSGRTFSSYTMGWFRQAPGKEREFVVAISKGGYKYDSVSLEARFTISKDNTKNTVYLQMNSLKPEDTAVYYCAATRAYGSSRLRLADTYEYWGQGTQVTVSSPDSEAAAKEAAAKEAAAKEAAAKEAAAKPDGSSQLQLVESGGGSVQPGGSLRLSCEVSGRTFSSYTMGWFRQAPGKEREFVVAISKGGYKYDSVSLEARFTISKDNTKNTVYLQMNSLKPEDTAVYYCAATRAYGSSRLRLADTYEYWGQGTQVTVSS

SEQ ID NO: 102 - protein, 259 aa, synthetic construct
QLQLVESGGGSVQPGGSLRLSCEVSGRTFASYTMGWFRQAPGKEREFVVAISKGGYKYDSVSLEARFTISKDNTKNTVYLQMNSLKPEDTAVYYCAGTRAYGSSRLRLAETYEYWGQGTQVTVSSSSSSSSSSSQLQLVESGGGSVQPGGSLRLSCEVSGRTFASYTMGWFRQAPGKEREFVVAISKGGYKYDSVSLEARFTISKDNTKNTVYLQMNSLKPEDTAVYYCAGTRAYGSSRLRLAETYEYWGQGTQVTVSS

SEQ ID NO: 103 - protein, 270 aa, synthetic construct
QLQLVESGGGSVQPGGSLRLSCEVSGRTFASYTMGWFRQAPGKEREFVVAISKGGYKYDSVSLEARFTISKDNTKNTVYLQMNSLKPEDTAVYYCAGTRAYGSSRLRLAETYEYWGQGTQVTVSSSSSSSSSSSSSSSSSSSSSSQLQLVESGGGSVQPGGSLRLSCEVSGRTFASYTMGWFRQAPGKEREFVVAISKGGYKYDSVSLEARFTISKDNTKNTVYLQMNSLKPEDTAVYYCAGTRAYGSSRLRLAETYEYWGQGTQVTVSS

SEQ ID NO: 104 - protein, 270 aa, synthetic construct
QLQLVESGGGSVQPGGSLRLSCEVSGRTFASYTMGWFRQAPGKEREFVVAISKGGYKYDSVSLEARFTISKDNTKNTVYLQMNSLKPEDTAVYYCAGTRAYGSSRLRLAETYEYWGQGTQVTVSSGGGGSGGGSGGGSGGGSGGSQLQLVESGGGSVQPGGSLRLSCEVSGRTFASYTMGWFRQAPGKEREFVVAISKGGYKYDSVSLEARFTISKDNTKNTVYLQMNSLKPEDTAVYYCAGTRAYGSSRLRLAETYEYWGQGTQVTVSS

SEQ ID NO: 105 - protein, 275 aa, synthetic construct
QLQLVESGGGSVQPGGSLRLSCEVSGRTFASYTMGWFRQAPGKEREFVVAISKGGYKYDSVSLEARFTISKDNTKNTVYLQMNSLKPEDTAVYYCAGTRAYGSSRLRLAETYEYWGQGTQVTVSSGGGGSGGGSGGGSGGGSGGGSGGGSQLQLVESGGGSVQPGGSLRLSCEVSGRTFASYTMGWFRQAPGKEREFVVAISKGGYKYDSVSLEARFTISKDNTKNTVYLQMNSLKPEDTAVYYCAGTRAYGSSRLRLAETYEYWGQGTQVTVSS

SEQ ID NO: 106 - protein, 280 aa, synthetic construct
QLQLVESGGGSVQPGGSLRLSCEVSGRTFASYTMGWFRQAPGKEREFVVAISKGGYKYDSVSLEARFTISKDNTKNTVYLQMNSLKPEDTAVYYCAGTRAYGSSRLRLAETYEYWGQGTQVTVSSGGGGSGGGSGGGGSGGGSGGGSGGGSGGGSQLQLVESGGGSVQPGGSLRLSCEVSGRTFASYTMGWFRQAPGKEREFVVAISKGGYKYDSVSLEARFTISKDNTKNTVYLQMNSLKPEDTAVYYCAGTRAYGSSRLRLAETYEYWGQGTQVTVSS

SEQ ID NO: 107 - protein, 289 aa, synthetic construct
QLQLVESGGGSVQPGGSLRLSCEVSGRTFASYTMGWFRQAPGKEREFVVAISKGGYKYDSVSLEARFTISKDNTKNTVYLQMNSLKPEDTAVYYCAGTRAYGSSRLRLAETYEYWGQGTQVTVSSGGGGSGGGSGGGGSGGGGSGGGGSGGGGSGGGGSGGGGSQLQLVESGGGSVQPGGSLRLSCEVSGRTFASYTMGWFRQAPGKEREFVVAISKGGYKYDSVSLEARFTISKDNTKNTVYLQMNSLKPEDTAVYYCAGTRAYGSSRLRLAETYEYWGQGTQVTVSS

SEQ ID NO: 108 - protein, 283 aa, synthetic construct
QLQLVESGGGSVQPGGSLRLSCEVSGRTFASYTMGWFRQAPGKEREFVVAISKGGYKYDSVSLEARFTISKDNTKNTVYLQMNSLKPEDTAVYYCAGTRAYGSSRLRLAETYEYWGQGTQVTVSSPDSEAAAKEAAAKEAAAKEAAAKEAAAKPDGSSQLQLVESGGGSVQPGGSLRLSCEVSGRTFASYTMGWFRQAPGKEREFVVAISKGGYKYDSVSLEARFTISKDNTKNTVYLQMNSLKPEDTAVYYCAGTRAYGSSRLRLAETYEYWGQGTQVTVSS

SEQ ID NO: 109 - protein, 250 aa, synthetic construct
EVQLVESGGGLVQPGGSLRLSCAVSGRTFSSYTMGWFRQAPGKEREFVVAISKGGYKYDSVSLEARFTISRDNAKNTVYLQMNSLRPEDTAVYYCAATRAYGSSRLRLADTYEYWGQGTLVTVSSEVQLVESGGGLVQPGGSLRLSCAVSGRTFSSYTMGWFRQAPGKEREFVVAISKGGYKYDSVSLEARFTISRDNAKNTVYLQMNSLRPEDTAVYYCAATRAYGSSRLRLADTYEYWGQGTLVTVSS

SEQ ID NO: 110 - protein, 253 aa, synthetic construct
EVQLVESGGGLVQPGGSLRLSCAVSGRTFSSYTMGWFRQAPGKEREFVVAISKGGYKYDSVSLEARFTISRDNAKNTVYLQMNSLRPEDTAVYYCAATRAYGSSRLRLADTYEYWGQGTLVTVSSGGSEVQLVESGGGLVQPGGSLRLSCAVSGRTFSSYTMGWFRQAPGKEREFVVAISKGGYKYDSVSLEARFTISRDNAKNTVYLQMNSLRPEDTAVYYCAATRAYGSSRLRLADTYEYWGQGTLVTVSS

SEQ ID NO: 111 - protein, 250 aa, synthetic construct
EVQLVESGGGLVQPGGSLRLSCAVSGRTFSSYTMGWFRQAPGKEREFVVAISKGGYKYDSVSLEARFTISRDNSKNTVYLQMNSLRPEDTAVYYCAATRAYGSSRLRLADTYEYWGQGTLVTVSSEVQLVESGGGLVQPGGSLRLSCAVSGRTFSSYTMGWFRQAPGKEREFVVAISKGGYKYDSVSLEARFTISRDNSKNTVYLQMNSLRPEDTAVYYCAATRAYGSSRLRLADTYEYWGQGTLVTVSS

SEQ ID NO: 112 - protein, 253 aa, synthetic construct
EVQLVESGGGLVQPGGSLRLSCAVSGRTFSSYTMGWFRQAPGKEREFVVAISKGGYKYDSVSLEARFTISRDNSKNTVYLQMNSLRPEDTAVYYCAATRAYGSSRLRLADTYEYWGQGTLVTVSSGGSEVQLVESGGGLVQPGGSLRLSCAVSGRTFSSYTMGWFRQAPGKEREFVVAISKGGYKYDSVSLEARFTISRDNSKNTVYLQMNSLRPEDTAVYYCAATRAYGSSRLRLADTYEYWGQGTLVTVSS

SEQ ID NO: 113 - protein, 259 aa, synthetic construct
EVQLVESGGGLVQPGGSLRLSCAVSGRTFSSYTMGWFRQAPGKEREFVVAISKGGYKYDSVSLEARFTISRDNSKNTVYLQMNSLRPEDTAVYYCAATRAYGSSRLRLADTYEYWGQGTLVTVSSGGGGSGGGSEVQLVESGGGLVQPGGSLRLSCAVSGRTFSSYTMGWFRQAPGKEREFVVAISKGGYKYDSVSLEARFTISRDNSKNTVYLQMNSLRPEDTAVYYCAATRAYGSSRLRLADTYEYWGQGTLVTVSS

SEQ ID NO: 114 - protein, 253 aa, synthetic construct
EVQLVESGGGLVQPGGSLRLSCAASGRTFSSYTMGWFRQAPGKEREFVVAISKGGYKYDSVSLEARFTISRDNSKNTVYLQMNSLRPEDTAVYYCAATRAYGSSRLRLADTYEYWGQGTLVTVSSGGSEVQLVESGGGLVQPGGSLRLSCAASGRTFSSYTMGWFRQAPGKEREFVVAISKGGYKYDSVSLEARFTISRDNSKNTVYLQMNSLRPEDTAVYYCAATRAYGSSRLRLADTYEYWGQGTLVTVSS

SEQ ID NO: 115 - protein, 253 aa, synthetic construct
EVQLVESGGGLVQPGGSLRLSCAASGRTFSSYTMGWFRQAPGKEREFVVAISKGGYKYDSVSLEARFTISRDNAKNTVYLQMNSLRPEDTAVYYCAATRAYGSSRLRLADTYEYWGQGTLVTVSSGGSEVQLVESGGGLVQPGGSLRLSCAASGRTFSSYTMGWFRQAPGKEREFVVAISKGGYKYDSVSLEARFTISRDNAKNTVYLQMNSLRPEDTAVYYCAATRAYGSSRLRLADTYEYWGQGTLVTVSS

SEQ ID NO: 116 - protein, 253 aa, synthetic construct
EVQLVESGGGLVQPGGSLRLSCAASGRTFSSYTMGWFRQAPGKEREFVVAISKGGYKYDSVSLEARFTISRDNAKNTVYLQMNSLRAEDTAVYYCAATRAYGSSRLRLADTYEYWGQGTLVTVSSGGSEVQLVESGGGLVQPGGSLRLSCAASGRTFSSYTMGWFRQAPGKEREFVVAISKGGYKYDSVSLEARFTISRDNAKNTVYLQMNSLRAEDTAVYYCAATRAYGSSRLRLADTYEYWGQGTLVTVSS

SEQ ID NO: 117 - protein, 250 aa, synthetic construct
EVQLVESGGGLVQPGGSLRLSCAASGRTFTSYTMGWFRQAPGKEREFVVAISKGGYKYDAVSLEARFTISRDNAKNTVYLQMNSLRPEDTAVYYCAGTRAYGSSRLRLADTYEYWGQGTLVTVSSEVQLVESGGGLVQPGGSLRLSCAASGRTFTSYTMGWFRQAPGKEREFVVAISKGGYKYDAVSLEARFTISRDNAKNTVYLQMNSLRPEDTAVYYCAGTRAYGSSRLRLADTYEYWGQGTLVTVSS

SEQ ID NO: 118 - protein, 253 aa, synthetic construct
EVQLVESGGGLVQPGGSLRLSCAASGRTFTSYTMGWFRQAPGKEREFVVAISKGGYKYDAVSLEARFTISRDNAKNTVYLQMNSLRPEDTAVYYCAGTRAYGSSRLRLADTYEYWGQGTLVTVSSGGSEVQLVESGGGLVQPGGSLRLSCAASGRTFTSYTMGWFRQAPGKEREFVVAISKGGYKYDAVSLEARFTISRDNAKNTVYLQMNSLRPEDTAVYYCAGTRAYGSSRLRLADTYEYWGQGTLVTVSS

SEQ ID NO: 119 - protein, 250 aa, synthetic construct
EVQLVESGGGLVQPGGSLRLSCAASGRTFASYTMGWFRQAPGKEREFVVAISKGGYKYDSVSLEARFTISRDNAKNTVYLQMNSLRPEDTAVYYCAGTRAYGSSRLRLAETYEYWGQGTLVTVSSEVQLVESGGGLVQPGGSLRLSCAASGRTFASYTMGWFRQAPGKEREFVVAISKGGYKYDSVSLEARFTISRDNAKNTVYLQMNSLRPEDTAVYYCAGTRAYGSSRLRLAETYEYWGQGTLVTVSS

SEQ ID NO: 120 - protein, 253 aa, synthetic construct
EVQLVESGGGLVQPGGSLRLSCAASGRTFASYTMGWFRQAPGKEREFVVAISKGGYKYDSVSLEARFTISRDNAKNTVYLQMNSLRPEDTAVYYCAGTRAYGSSRLRLAETYEYWGQGTLVTVSSGGSEVQLVESGGGLVQPGGSLRLSCAASGRTFASYTMGWFRQAPGKEREFVVAISKGGYKYDSVSLEARFTISRDNAKNTVYLQMNSLRPEDTAVYYCAGTRAYGSSRLRLAETYEYWGQGTLVTVSS

SEQ ID NO: 121 - protein, 250 aa, synthetic construct
EVQLVESGGGLVQPGGSLRLSCAASGRTFSSYTMGWFRQAPGKEREFVVAISKGGYKYDAVSLEARFTISRDNSKNTVYLQMNSLRPEDTAVYYCAATRAYGSSRLRLAKTYEYWGQGTLVTVSSEVQLVESGGGLVQPGGSLRLSCAASGRTFSSYTMGWFRQAPGKEREFVVAISKGGYKYDAVSLEARFTISRDNSKNTVYLQMNSLRPEDTAVYYCAATRAYGSSRLRLAKTYEYWGQGTLVTVSS

SEQ ID NO: 122 - protein, 253 aa, synthetic construct
EVQLVESGGGLVQPGGSLRLSCAASGRTFSSYTMGWFRQAPGKEREFVVAISKGGYKYDAVSLEARFTISRDNSKNTVYLQMNSLRPEDTAVYYCAATRAYGSSRLRLAKTYEYWGQGTLVTVSSGGSEVQLVESGGGLVQPGGSLRLSCAASGRTFSSYTMGWFRQAPGKEREFVVAISKGGYKYDAVSLEARFTISRDNSKNTVYLQMNSLRPEDTAVYYCAATRAYGSSRLRLAKTYEYWGQGTLVTVSS

SEQ ID NO: 123 - protein, 250 aa, synthetic construct
EVQLVESGGGLVQPGGSLRLSCAASGRTFSSYTMGWFRQAPGKGREFVVAISKGGYKYDAVSLEARFTISRDNSKNTVYLQMNSLRPEDTAVYYCAATRAYGSSRLRLAKTYEYWGQGTLVTVSSEVQLVESGGGLVQPGGSLRLSCAASGRTFSSYTMGWFRQAPGKGREFVVAISKGGYKYDAVSLEARFTISRDNSKNTVYLQMNSLRPEDTAVYYCAATRAYGSSRLRLAKTYEYWGQGTLVTVSS

SEQ ID NO: 124 - protein, 253 aa, synthetic construct
EVQLVESGGGLVQPGGSLRLSCAASGRTFSSYTMGWFRQAPGKGREFVVAISKGGYKYDAVSLEARFTISRDNSKNTVYLQMNSLRPEDTAVYYCAATRAYGSSRLRLAKTYEYWGQGTLVTVSSGGSEVQLVESGGGLVQPGGSLRLSCAASGRTFSSYTMGWFRQAPGKGREFVVAISKGGYKYDAVSLEARFTISRDNSKNTVYLQMNSLRPEDTAVYYCAATRAYGSSRLRLAKTYEYWGQGTLVTVSS

SEQ ID NO: 125 - protein, 259 aa, synthetic construct
EVQLVESGGGLVQPGGSLRLSCAASGRTFSSYTMGWFRQAPGKGREFVVAISKGGYKYDAVSLEARFTISRDNSKNTVYLQMNSLRPEDTAVYYCAATRAYGSSRLRLAKTYEYWGQGTLVTVSSGGGGSGGGSEVQLVESGGGLVQPGGSLRLSCAASGRTFSSYTMGWFRQAPGKGREFVVAISKGGYKYDAVSLEARFTISRDNSKNTVYLQMNSLRPEDTAVYYCAATRAYGSSRLRLAKTYEYWGQGTLVTVSS

SEQ ID NO: 126 - protein, 250 aa, synthetic construct
EVQLVESGGGLVQPGGSLRLSCAASGRTFSSYTMGWFRQAPGKEREFVVAISKGGYKYNAVSLEARFTISRDNSKNTVYLQMNSLRPEDTAVYYCAATRAYGSSRLRLAKTYEYWGQGTLVTVSSEVQLVESGGGLVQPGGSLRLSCAASGRTFSSYTMGWFRQAPGKEREFVVAISKGGYKYNAVSLEARFTISRDNSKNTVYLQMNSLRPEDTAVYYCAATRAYGSSRLRLAKTYEYWGQGTLVTVSS

SEQ ID NO: 127 - protein, 253 aa, synthetic construct
EVQLVESGGGLVQPGGSLRLSCAASGRTFSSYTMGWFRQAPGKEREFVVAISKGGYKYNAVSLEARFTISRDNSKNTVYLQMNSLRPEDTAVYYCAATRAYGSSRLRLAKTYEYWGQGTLVTVSSGGSEVQLVESGGGLVQPGGSLRLSCAASGRTFSSYTMGWFRQAPGKEREFVVAISKGGYKYNAVSLEARFTISRDNSKNTVYLQMNSLRPEDTAVYYCAATRAYGSSRLRLAKTYEYWGQGTLVTVSS

SEQ ID NO: 128 - protein, 259 aa, synthetic construct
EVQLVESGGGLVQPGGSLRLSCAASGRTFSSYTMGWFRQAPGKEREFVVAISKGGYKYNAVSLEARFTISRDNSKNTVYLQMNSLRPEDTAVYYCAATRAYGSSRLRLAKTYEYWGQGTLVTVSSGGGGSGGGSEVQLVESGGGLVQPGGSLRLSCAASGRTFSSYTMGWFRQAPGKEREFVVAISKGGYKYNAVSLEARFTISRDNSKNTVYLQMNSLRPEDTAVYYCAATRAYGSSRLRLAKTYEYWGQGTLVTVSS

SEQ ID NO: 129 - protein, 250 aa, synthetic construct
EVQLVESGGGLVQPGGSLRLSCAASGRTFSSYTMGWFRQAPGKEREFVVAISKGGYKYNAVSLEARFTISRDNAKNTVYLQMNSLRPEDTAVYYCASTRAYGSSRLRLAKTYEYWGQGTLVTVSSEVQLVESGGGLVQPGGSLRLSCAASGRTFSSYTMGWFRQAPGKEREFVVAISKGGYKYNAVSLEARFTISRDNAKNTVYLQMNSLRPEDTAVYYCASTRAYGSSRLRLAKTYEYWGQGTLVTVSS

SEQ ID NO: 130 - protein, 253 aa, synthetic construct
EVQLVESGGGLVQPGGSLRLSCAASGRTFSSYTMGWFRQAPGKEREFVVAISKGGYKYNAVSLEARFTISRDNAKNTVYLQMNSLRPEDTAVYYCASTRAYGSSRLRLAKTYEYWGQGTLVTVSSGGSEVQLVESGGGLVQPGGSLRLSCAASGRTFSSYTMGWFRQAPGKEREFVVAISKGGYKYNAVSLEARFTISRDNAKNTVYLQMNSLRPEDTAVYYCASTRAYGSSRLRLAKTYEYWGQGTLVTVSS

SEQ ID NO: 131 - protein, 259 aa, synthetic construct
EVQLVESGGGLVQPGGSLRLSCAASGRTFSSYTMGWFRQAPGKEREFVVAISKGGYKYNAVSLEARFTISRDNAKNTVYLQMNSLRPEDTAVYYCASTRAYGSSRLRLAKTYEYWGQGTLVTVSSGGGGSGGGSEVQLVESGGGLVQPGGSLRLSCAASGRTFSSYTMGWFRQAPGKEREFVVAISKGGYKYNAVSLEARFTISRDNAKNTVYLQMNSLRPEDTAVYYCASTRAYGSSRLRLAKTYEYWGQGTLVTVSS

SEQ ID NO: 132 - protein, 250 aa, synthetic construct
EVQLVESGGGLVQPGGSLRLSCAASGRTFSSYTMGWFRQAPGKEREFVVAISKGGYKYDSVSLEARFTISRDNSKNTVYLQMNSLRPEDTAVYYCAATRAYGSSRLRLANTYEYWGQGTLVTVSSEVQLVESGGGLVQPGGSLRLSCAASGRTFSSYTMGWFRQAPGKEREFVVAISKGGYKYDSVSLEARFTISRDNSKNTVYLQMNSLRPEDTAVYYCAATRAYGSSRLRLANTYEYWGQGTLVTVSS

SEQ ID NO: 133 - protein, 253 aa, synthetic construct
EVQLVESGGGLVQPGGSLRLSCAASGRTFSSYTMGWFRQAPGKEREFVVAISKGGYKYDSVSLEARFTISRDNSKNTVYLQMNSLRPEDTAVYYCAATRAYGSSRLRLANTYEYWGQGTLVTVSSGGSEVQLVESGGGLVQPGGSLRLSCAASGRTFSSYTMGWFRQAPGKEREFVVAISKGGYKYDSVSLEARFTISRDNSKNTVYLQMNSLRPEDTAVYYCAATRAYGSSRLRLANTYEYWGQGTLVTVSS

SEQ ID NO: 134 - protein, 227 aa, synthetic construct
DKTHTCPPCPAPELLGGPSVFLFPPKPKDTLMISRTPEVTCVVVDVSHEDPEVKFNWYVDGVEVHNAKTKPREEQYNSTYRVVSVLTVLHQDWLNGKEYKCKVSNKALPAPIEKTISKAKGQPREPQVYTLPPSRDELTKNQVSLTCLVKGFYPSDIAVEWESNGQPENNYKTTPPVLDSDGSFFLYSKLTVDKSRWQQGNVFSCSVMHEALHNHYTQKSLSLSPGK

SEQ ID NO: 135 - protein, 227 aa, synthetic construct
DKTHTCPPCPAPELLGGPSVFLFPPKPKDTLMISRTPEVTCVVVDVSHEDPEVKFNWYVDGVEVHNAKTKPREEQYNSTYRVVSVLTVLHQDWLNGKEYKCKVSNKALPAPIEKTISKAKGQPREPQVYTLPPSREEMTKNQVSLTCLVKGFYPSDIAVEWESNGQPENNYKTTPPVLDSDGSFFLYSKLTVDKSRWQQGNVFSCSVMHEALHNHYTQKSLSLSPGK

SEQ ID NO: 136 - protein, 346 aa, synthetic construct
QLQLVESGGGSVQPGGSLRLSCEVSGRTFASYTMGWFRQAPGKEREFVVAISKGGYKYDSVSLEARFTISKDNTKNTVYLQMNSLKPEDTAVYYCAGTRAYGSSRLRLAETYEYWGQGTQVTVSSPPCPAPELLGGPSVFLFPPKPKDTLMISRTPEVTCVVVDVSHEDPEVKFNWYVDGVEVHNAKTKPREEQYNSTYRVVSVLTVLHQDWLNGKEYKCKVSNKALPAPIEKTISKAKGQPREPQVYTLPPSRDELTKNQVSLTCLVKGFYPSDIAVEWESNGQPENNYKTTPPVLDSDGSFFLYSKLTVDKSRWQQGNVFSCSVMHEALHNHYTQKSLSLSPGK

SEQ ID NO: 137 - protein, 355 aa, synthetic construct
QLQLVESGGGSVQPGGSLRLSCEVSGRTFASYTMGWFRQAPGKEREFVVAISKGGYKYDSVSLEARFTISKDNTKNTVYLQMNSLKPEDTAVYYCAGTRAYGSSRLRLAETYEYWGQGTQVTVSSGGGGSGGGSPPCPAPELLGGPSVFLFPPKPKDTLMISRTPEVTCVVVDVSHEDPEVKFNWYVDGVEVHNAKTKPREEQYNSTYRVVSVLTVLHQDWLNGKEYKCKVSNKALPAPIEKTISKAKGQPREPQVYTLPPSRDELTKNQVSLTCLVKGFYPSDIAVEWESNGQPENNYKTTPPVLDSDGSFFLYSKLTVDKSRWQQGNVFSCSVMHEALHNHYTQKSLSLSPGK

SEQ ID NO: 138 - protein, 352 aa, synthetic construct
QLQLVESGGGSVQPGGSLRLSCEVSGRTFASYTMGWFRQAPGKEREFVVAISKGGYKYDSVSLEARFTISKDNTKNTVYLQMNSLKPEDTAVYYCAGTRAYGSSRLRLAETYEYWGQGTQVTVSSDKTHTCPPCPAPELLGGPSVFLFPPKPKDTLMISRTPEVTCVVVDVSHEDPEVKFNWYVDGVEVHNAKTKPREEQYNSTYRVVSVLTVLHQDWLNGKEYKCKVSNKALPAPIEKTISKAKGQPREPQVYTLPPSRDELTKNQVSLTCLVKGFYPSDIAVEWESNGQPENNYKTTPPVLDSDGSFFLYSKLTVDKSRWQQGNVFSCSVMHEALHNHYTQKSLSLSPGK

SEQ ID NO: 139 - protein, 357 aa, synthetic construct
EVQLVESGGGLVQPGGSLRLSCAVSGRTFSSYTMGWFRQAPGKEREFVVAISKGGYKYDSVSLEARFTISRDNAKNTVYLQMNSLRPEDTAVYYCAATRAYGSSRLRLADTYEYWGQGTLVTVSSEPKSADKTHTCPPCPAPELLGGPSVFLFPPKPKDTLMISRTPEVTCVVVDVSHEDPEVKFNWYVDGVEVHNAKTKPREEQYNSTYRVVSVLTVLHQDWLNGKEYKCKVSNKALPAPIEKTISKAKGQPREPQVYTLPPSREEMTKNQVSLTCLVKGFYPSDIAVEWESNGQPENNYKTTPPVLDSDGSFFLYSKLTVDKSRWQQGNVFSCSVMHEALHNHYTQKSLSLSPGK

SEQ ID NO: 140 - protein, 477 aa, synthetic construct
EVQLVESGGGLVQPGGSLRLSCAVSGRTFSSYTMGWFRQAPGKEREFVVAISKGGYKYDSVSLEARFTISRDNAKNTVYLQMNSLRPEDTAVYYCAATRAYGSSRLRLADTYEYWGQGTLVTVSSEVQLVESGGGLVQPGGSLRLSCAVSGRTFSSYTMGWFRQAPGKEREFVVAISKGGYKYDSVSLEARFTISRDNAKNTVYLQMNSLRPEDTAVYYCAATRAYGSSRLRLADTYEYWGQGTLVTVSSDKTHTCPPCPAPELLGGPSVFLFPPKPKDTLMISRTPEVTCVVVDVSHEDPEVKFNWYVDGVEVHNAKTKPREEQYNSTYRVVSVLTVLHQDWLNGKEYKCKVSNKALPAPIEKTISKAKGQPREPQVYTLPPSRDELTKNQVSLTCLVKGFYPSDIAVEWESNGQPENNYKTTPPVLDSDGSFFLYSKLTVDKSRWQQGNVFSCSVMHEALHNHYTQKSLSLSPGK

SEQ ID NO: 141 - protein, 480 aa, synthetic construct
EVQLVESGGGLVQPGGSLRLSCAVSGRTFSSYTMGWFRQAPGKEREFVVAISKGGYKYDSVSLEARFTISRDNAKNTVYLQMNSLRPEDTAVYYCAATRAYGSSRLRLADTYEYWGQGTLVTVSSGGSEVQLVESGGGLVQPGGSLRLSCAVSGRTFSSYTMGWFRQAPGKEREFVVAISKGGYKYDSVSLEARFTISRDNAKNTVYLQMNSLRPEDTAVYYCAATRAYGSSRLRLADTYEYWGQGTLVTVSSDKTHTCPPCPAPELLGGPSVFLFPPKPKDTLMISRTPEVTCVVVDVSHEDPEVKFNWYVDGVEVHNAKTKPREEQYNSTYRVVSVLTVLHQDWLNGKEYKCKVSNKALPAPIEKTISKAKGQPREPQVYTLPPSRDELTKNQVSLTCLVKGFYPSDIAVEWESNGQPENNYKTTPPVLDSDGSFFLYSKLTVDKSRWQQGNVFSCSVMHEALHNHYTQKSLSLSPGK

SEQ ID NO: 142 - protein, 480 aa, synthetic construct
EVQLVESGGGLVQPGGSLRLSCAVSGRTFSSYTMGWFRQAPGKEREFVVAISKGGYKYDSVSLEARFTISRDNSKNTVYLQMNSLRPEDTAVYYCAATRAYGSSRLRLADTYEYWGQGTLVTVSSGGSEVQLVESGGGLVQPGGSLRLSCAVSGRTFSSYTMGWFRQAPGKEREFVVAISKGGYKYDSVSLEARFTISRDNSKNTVYLQMNSLRPEDTAVYYCAATRAYGSSRLRLADTYEYWGQGTLVTVSSDKTHTCPPCPAPELLGGPSVFLFPPKPKDTLMISRTPEVTCVVVDVSHEDPEVKFNWYVDGVEVHNAKTKPREEQYNSTYRVVSVLTVLHQDWLNGKEYKCKVSNKALPAPIEKTISKAKGQPREPQVYTLPPSRDELTKNQVSLTCLVKGFYPSDIAVEWESNGQPENNYKTTPPVLDSDGSFFLYSKLTVDKSRWQQGNVFSCSVMHEALHNHYTQKSLSLSPGK

SEQ ID NO: 143 - protein, 486 aa, synthetic construct
EVQLVESGGGLVQPGGSLRLSCAVSGRTFSSYTMGWFRQAPGKEREFVVAISKGGYKYDSVSLEARFTISRDNSKNTVYLQMNSLRPEDTAVYYCAATRAYGSSRLRLADTYEYWGQGTLVTVSSGGGGSGGGSEVQLVESGGGLVQPGGSLRLSCAVSGRTFSSYTMGWFRQAPGKEREFVVAISKGGYKYDSVSLEARFTISRDNSKNTVYLQMNSLRPEDTAVYYCAATRAYGSSRLRLADTYEYWGQGTLVTVSSDKTHTCPPCPAPELLGGPSVFLFPPKPKDTLMISRTPEVTCVVVDVSHEDPEVKFNWYVDGVEVHNAKTKPREEQYNSTYRVVSVLTVLHQDWLNGKEYKCKVSNKALPAPIEKTISKAKGQPREPQVYTLPPSRDELTKNQVSLTCLVKGFYPSDIAVEWESNGQPENNYKTTPPVLDSDGSFFLYSKLTVDKSRWQQGNVFSCSVMHEALHNHYTQKSLSLSPGK

SEQ ID NO: 144 - protein, 480 aa, synthetic construct
EVQLVESGGGLVQPGGSLRLSCAASGRTFSSYTMGWFRQAPGKEREFVVAISKGGYKYDSVSLEARFTISRDNSKNTVYLQMNSLRPEDTAVYYCAATRAYGSSRLRLADTYEYWGQGTLVTVSSGGSEVQLVESGGGLVQPGGSLRLSCAASGRTFSSYTMGWFRQAPGKEREFVVAISKGGYKYDSVSLEARFTISRDNSKNTVYLQMNSLRPEDTAVYYCAATRAYGSSRLRLADTYEYWGQGTLVTVSSDKTHTCPPCPAPELLGGPSVFLFPPKPKDTLMISRTPEVTCVVVDVSHEDPEVKFNWYVDGVEVHNAKTKPREEQYNSTYRVVSVLTVLHQDWLNGKEYKCKVSNKALPAPIEKTISKAKGQPREPQVYTLPPSRDELTKNQVSLTCLVKGFYPSDIAVEWESNGQPENNYKTTPPVLDSDGSFFLYSKLTVDKSRWQQGNVFSCSVMHEALHNHYTQKSLSLSPGK

SEQ ID NO: 145 - protein, 480 aa, synthetic construct
EVQLVESGGGLVQPGGSLRLSCAASGRTFSSYTMGWFRQAPGKEREFVVAISKGGYKYDSVSLEARFTISRDNAKNTVYLQMNSLRPEDTAVYYCAATRAYGSSRLRLADTYEYWGQGTLVTVSSGGSEVQLVESGGGLVQPGGSLRLSCAASGRTFSSYTMGWFRQAPGKEREFVVAISKGGYKYDSVSLEARFTISRDNAKNTVYLQMNSLRPEDTAVYYCAATRAYGSSRLRLADTYEYWGQGTLVTVSSDKTHTCPPCPAPELLGGPSVFLFPPKPKDTLMISRTPEVTCVVVDVSHEDPEVKFNWYVDGVEVHNAKTKPREEQYNSTYRVVSVLTVLHQDWLNGKEYKCKVSNKALPAPIEKTISKAKGQPREPQVYTLPPSRDELTKNQVSLTCLVKGFYPSDIAVEWESNGQPENNYKTTPPVLDSDGSFFLYSKLTVDKSRWQQGNVFSCSVMHEALHNHYTQKSLSLSPGK

SEQ ID NO: 146 - protein, 477 aa, synthetic construct
EVQLVESGGGLVQPGGSLRLSCAASGRTFTSYTMGWFRQAPGKEREFVVAISKGGYKYDAVSLEARFTISRDNAKNTVYLQMNSLRPEDTAVYYCAGTRAYGSSRLRLADTYEYWGQGTLVTVSSEVQLVESGGGLVQPGGSLRLSCAASGRTFTSYTMGWFRQAPGKEREFVVAISKGGYKYDAVSLEARFTISRDNAKNTVYLQMNSLRPEDTAVYYCAGTRAYGSSRLRLADTYEYWGQGTLVTVSSDKTHTCPPCPAPELLGGPSVFLFPPKPKDTLMISRTPEVTCVVVDVSHEDPEVKFNWYVDGVEVHNAKTKPREEQYNSTYRVVSVLTVLHQDWLNGKEYKCKVSNKALPAPIEKTISKAKGQPREPQVYTLPPSRDELTKNQVSLTCLVKGFYPSDIAVEWESNGQPENNYKTTPPVLDSDGSFFLYSKLTVDKSRWQQGNVFSCSVMHEALHNHYTQKSLSLSPGK

SEQ ID NO: 147 - protein, 480 aa, synthetic construct
EVQLVESGGGLVQPGGSLRLSCAASGRTFASYTMGWFRQAPGKEREFVVAISKGGYKYDSVSLEARFTISRDNAKNTVYLQMNSLRPEDTAVYYCAGTRAYGSSRLRLAETYEYWGQGTLVTVSSGGSEVQLVESGGGLVQPGGSLRLSCAASGRTFASYTMGWFRQAPGKEREFVVAISKGGYKYDSVSLEARFTISRDNAKNTVYLQMNSLRPEDTAVYYCAGTRAYGSSRLRLAETYEYWGQGTLVTVSSDKTHTCPPCPAPELLGGPSVFLFPPKPKDTLMISRTPEVTCVVVDVSHEDPEVKFNWYVDGVEVHNAKTKPREEQYNSTYRVVSVLTVLHQDWLNGKEYKCKVSNKALPAPIEKTISKAKGQPREPQVYTLPPSRDELTKNQVSLTCLVKGFYPSDIAVEWESNGQPENNYKTTPPVLDSDGSFFLYSKLTVDKSRWQQGNVFSCSVMHEALHNHYTQKSLSLSPGK

SEQ ID NO: 148 - protein, 480 aa, synthetic construct
EVQLVESGGGLVQPGGSLRLSCAASGRTFSSYTMGWFRQAPGKEREFVVAISKGGYKYDAVSLEARFTISRDNSKNTVYLQMNSLRPEDTAVYYCAATRAYGSSRLRLAKTYEYWGQGTLVTVSSGGSEVQLVESGGGLVQPGGSLRLSCAASGRTFSSYTMGWFRQAPGKEREFVVAISKGGYKYDAVSLEARFTISRDNSKNTVYLQMNSLRPEDTAVYYCAATRAYGSSRLRLAKTYEYWGQGTLVTVSSDKTHTCPPCPAPELLGGPSVFLFPPKPKDTLMISRTPEVTCVVVDVSHEDPEVKFNWYVDGVEVHNAKTKPREEQYNSTYRVVSVLTVLHQDWLNGKEYKCKVSNKALPAPIEKTISKAKGQPREPQVYTLPPSRDELTKNQVSLTCLVKGFYPSDIAVEWESNGQPENNYKTTPPVLDSDGSFFLYSKLTVDKSRWQQGNVFSCSVMHEALHNHYTQKSLSLSPGK

SEQ ID NO: 149 - protein, 480 aa, synthetic construct
EVQLVESGGGLVQPGGSLRLSCAASGRTFSSYTMGWFRQAPGKGREFVVAISKGGYKYDAVSLEARFTISRDNSKNTVYLQMNSLRPEDTAVYYCAATRAYGSSRLRLAKTYEYWGQGTLVTVSSGGSEVQLVESGGGLVQPGGSLRLSCAASGRTFSSYTMGWFRQAPGKGREFVVAISKGGYKYDAVSLEARFTISRDNSKNTVYLQMNSLRPEDTAVYYCAATRAYGSSRLRLAKTYEYWGQGTLVTVSSDKTHTCPPCPAPELLGGPSVFLFPPKPKDTLMISRTPEVTCVVVDVSHEDPEVKFNWYVDGVEVHNAKTKPREEQYNSTYRVVSVLTVLHQDWLNGKEYKCKVSNKALPAPIEKTISKAKGQPREPQVYTLPPSRDELTKNQVSLTCLVKGFYPSDIAVEWESNGQPENNYKTTPPVLDSDGSFFLYSKLTVDKSRWQQGNVFSCSVMHEALHNHYTQKSLSLSPGK

SEQ ID NO: 150 - protein, 483 aa, synthetic construct
EVQLVESGGGLVQPGGSLRLSCAASGRTFSSYTMGWFRQAPGKGREFVVAISKGGYKYDAVSLEARFTISRDNSKNTVYLQMNSLRPEDTAVYYCAATRAYGSSRLRLAKTYEYWGQGTLVTVSSGGSGGSEVQLVESGGGLVQPGGSLRLSCAASGRTFSSYTMGWFRQAPGKGREFVVAISKGGYKYDAVSLEARFTISRDNSKNTVYLQMNSLRPEDTAVYYCAATRAYGSSRLRLAKTYEYWGQGTLVTVSSDKTHTCPPCPAPELLGGPSVFLFPPKPKDTLMISRTPEVTCVVVDVSHEDPEVKFNWYVDGVEVHNAKTKPREEQYNSTYRVVSVLTVLHQDWLNGKEYKCKVSNKALPAPIEKTISKAKGQPREPQVYTLPPSRDELTKNQVSLTCLVKGFYPSDIAVEWESNGQPENNYKTTPPVLDSDGSFFLYSKLTVDKSRWQQGNVFSCSVMHEALHNHYTQKSLSLSPGK

SEQ ID NO: 151 - protein, 23 aa, synthetic construct
MDAMKRGLCCVLLLCGAVFVSPS

SEQ ID NO: 152 - protein, 5 aa, synthetic construct
GGGGS

SEQ ID NO: 153 - protein, 4 aa, synthetic construct
SGGS

SEQ ID NO: 154 - protein, 6 aa, synthetic construct
HHHHHH

SEQ ID NO: 155 - protein, 20 aa, synthetic construct
METDTLLLWVLLLWVPGSTG

SEQ ID NO: 156 - protein, 5 aa, synthetic construct
EPKSA

SEQ ID NO: 157 - protein, 121 aa, synthetic construct
APMAEEGDNKPHEVVKFMEVYRRSYCQPIETLVDIFQEYPDEIEYIFKPSCVPLVRCGGCCNDESLECVPTEEFNVTMQIMRIKPHQGQHIGEMSFLQHNKCECRPKKDRARQEKCDKPRR

SEQ ID NO: 158 - protein, 221 aa, synthetic construct
PPCPAPELLGGPSVFLFPPKPKDTLMISRTPEVTCVVVDVSHEDPEVKFNWYVDGVEVHNAKTKPREEQYNSTYRVVSVLTVLHQDWLNGKEYKCKVSNKALPAPIEKTISKAKGQPREPQVYTLPPSRDELTKNQVSLTCLVKGFYPSDIAVEWESNGQPENNYKTTPPVLDSDGSFFLYSKLTVDKSRWQQGNVFSCSVMHEALHNHYTQKSLSLSPGK

SEQ ID NO: 159 - protein, 287 aa, synthetic construct
QLQLVESGGGSVQPGGSLRLSCEVSGRTFSSYTMGWFRQAPGKEREFVVAISKGGYKYDSVSLEARFTISKDNTKNTVYLQMNSLKPEDTAVYYCAATRAYGSSRLRLADTYEYWGQGTQVTVSSGSTSGSGKPGSGEGSTKGGSTSGSGKPGSGEGSTKGSQLQLVESGGGSVQPGGSLRLSCEVSGRTFSSYTMGWFRQAPGKEREFVVAISKGGYKYDSVSLEARFTISKDNTKNTVYLQMNSLKPEDTAVYYCAATRAYGSSRLRLADTYEYWGQGTQVTVSS